European Patent Specification EP 3 985 101 B1, published April 23, 2025. Title: Method for producing a medium composition for culturing adherent cells in suspension. Applicant: NISSAN CHEMICAL CORPORATION. The sequence listing filed with the application follows.

SEQUENCE LISTING (3 sequences)

SEQ ID NO: 1 - protein, 417 aa, Artificial Sequence
  amino acid fragment of 62-478 of human vitronectin
VTRGDVFTMPEDEYTVYDDGEEKNNATVHEQVGGPSLTSDLQAQSKGNPEQTPVLKPEEEAPAPEVGASKPEGIDSRPETLHPGRPQPPAEEELCSGKPFDAFTDLKNGSLFAFRGQYCYELDEKAVRPGYPKLIRDVWGIEGPIDAAFTRINCQGKTYLFKGSQYWRFEDGVLDPDYPRNISDGFDGIPDNVDAALALPAHSYSGRERVYFFKGKQYWEYQFQHQPSQEECEGSSLSAVFEHFAMMQRDSWEDIFELLFWGRTSAGTRQPQFISRDWHGVPGQVDAAMAGRIYISGMAPRPSLAKKQRFRHRNRKGYRSQRGHSRGRNQNSRRPSRAMWLSLFSSEESNLGANNYDDYRMDWLVPATCEPIQSVFFFSGDKYYRVNLRTRRVDTVDPPYPRSIAQYWLGCPAPGHL

SEQ ID NO: 2 - protein, 379 aa, Artificial Sequence
  amino acid fragment of 20 to 398 of human vitronectin
DQESCKGRCTEGFNVDKKCQCDELCSYYQSCCTDYTAECKPQVTRGDVFTMPEDEYTVYDDGEEKNNATVHEQVGGPSLTSDLQAQSKGNPEQTPVLKPEEEAPAPEVGASKPEGIDSRPETLHPGRPQPPAEEELCSGKPFDAFTDLKNGSLFAFRGQYCYELDEKAVRPGYPKLIRDVWGIEGPIDAAFTRINCQGKTYLFKGSQYWRFEDGVLDPDYPRNISDGFDGIPDNVDAALALPAHSYSGRERVYFFKGKQYWEYQFQHQPSQEECEGSSLSAVFEHFAMMQRDSWEDIFELLFWGRTSAGTRQPQFISRDWHGVPGQVDAAMAGRIYISGMAPRPSLAKKQRFRHRNRKGYRSQRGHSRGRNQNSRRPSR

SEQ ID NO: 3 - protein, 459 aa, Artificial Sequence
  amino acid fragment of 20-478 of human vitronectin
DQESCKGRCTEGFNVDKKCQCDELCSYYQSCCTDYTAECKPQVTRGDVFTMPEDEYTVYDDGEEKNNATVHEQVGGPSLTSDLQAQSKGNPEQTPVLKPEEEAPAPEVGASKPEGIDSRPETLHPGRPQPPAEEELCSGKPFDAFTDLKNGSLFAFRGQYCYELDEKAVRPGYPKLIRDVWGIEGPIDAAFTRINCQGKTYLFKGSQYWRFEDGVLDPDYPRNISDGFDGIPDNVDAALALPAHSYSGRERVYFFKGKQYWEYQFQHQPSQEECEGSSLSAVFEHFAMMQRDSWEDIFELLFWGRTSAGTRQPQFISRDWHGVPGQVDAAMAGRIYISGMAPRPSLAKKQRFRHRNRKGYRSQRGHSRGRNQNSRRPSRAMWLSLFSSEESNLGANNYDDYRMDWLVPATCEPIQSVFFFSGDKYYRVNLRTRRVDTVDPPYPRSIAQYWLGCPAPGHL